European Patent Specification EP 3 280 799 B1, published October 30, 2024. Title: PRODUCTION OF OVERSIZED ADENO-ASSOCIATED VECTORS. Applicant: KYOSTIO-MOORE, Sirkka SOUZA, David VINCENT, Karen. Application Not Yet Assigned. The sequence listing filed with the application follows.

SEQUENCE LISTING (24 sequences)

SEQ ID NO: 1 - DNA, 5097 bp, Artificial Sequence
  Synthetic Construct
gagctcttggccactccctctctgcgcgctcgctcgctcactgaggccgggcgaccaaaggtcgcccgacgcccgggctttgcccgggcggcctcagtgagcgagcgagcgcgcagagagggagtggccaactccatcactaggggttcctacgcgtgtctgtctgcacatttcgtagagcgagtgttccgatactctaatctccctaggcaaggttcatatttgtgtaggttacttattctccttttgttgactaagtcaataatcagaatcagcaggtttggagtcagcttggcagggatcagcagcctgggttggaaggagggggtataaaagccccttcaccaggagaagccgtcacacagatccacaagctcctgctagcaggtaagtgccgtgtgtggttcccgcgggcctggcctctttacgggttatggcccttgcgtgccttgaattactgacactgacatccactttttctttttctccacaggtatcgattctctagagccaccatgcagatcgagctgtctacctgcttcttcctgtgcctgctgcggttctgcttcagcgccaccagacggtactatctgggcgccgtggaactgagctgggactacatgcagagcgacctgggcgagctgcccgtggatgccagattccctccaagagtgcccaagagcttccccttcaacacctccgtggtgtacaagaaaaccctgttcgtggaattcaccgaccacctgttcaatatcgccaagcccagacccccctggatgggcctgctgggacctacaattcaggccgaggtgtacgacaccgtcgtgatcaccctgaagaacatggccagccaccccgtgtctctgcatgccgtgggagtgtcctactggaaggcctctgagggcgccgagtacgacgatcagaccagccagcgcgagaaagaggacgacaaggtgttccctggcggcagccacacctacgtgtggcaggtgctgaaagaaaacggccccatggcctccgaccctctgtgcctgacatacagctacctgagccacgtggacctcgtgaaggacctgaacagcggcctgatcggagccctgctcgtgtgtagagagggcagcctggccaaagagaaaacccagaccctgcacaagttcatcctgctgttcgccgtgttcgacgagggcaagagctggcacagcgagacaaagaacagcctgatgcaggaccgggacgccgcctctgctagagcctggcccaaaatgcacaccgtgaacggctacgtgaacagaagcctgcccggactgatcggctgccaccggaagtctgtgtactggcacgtgatcggcatgggcaccacccctgaggtgcacagcatctttctggaaggacacacctttctcgtgcggaaccaccggcaggccagcctggaaatcagccctatcaccttcctgaccgcccagacactgctgatggacctgggccagtttctgctgttctgccacatcagctcccaccagcacgacggcatggaagcctacgtgaaggtggacagctgccccgaggaaccccagctgcggatgaagaacaacgaggaagccgaggactacgacgacgacctgaccgacagcgagatggacgtggtgcgcttcgacgacgataacagccccagcttcatccagatcagaagcgtggccaagaagcaccccaagacctgggtgcactatatcgccgccgaggaagaggactgggattacgcccctctggtgctggcccccgacgacagaagctacaagagccagtacctgaacaatggcccccagcggatcggccggaagtataagaaagtgcggttcatggcctacaccgacgagacattcaagaccagagaggccatccagcacgagagcggcatcctgggccctctgctgtatggcgaagtgggcgacaccctgctgatcatcttcaagaaccaggccagcagaccctacaacatctaccctcacggcatcaccgacgtgcggcccctgtactccagaaggctgcccaagggcgtgaaacacctgaaggacttccccatcctgcccggcgagatcttcaagtacaagtggaccgtgaccgtggaagatggccccaccaagagcgaccccagatgcctgacacggtactacagcagcttcgtgaacatggaacgggacctggcctccggcctgattggcccactgctgatctgctacaaagaaagcgtggaccagcggggcaaccagatcatgagcgacaagcggaacgtgatcctgtttagcgtgttcgatgagaaccggtcctggtatctgaccgagaatatccagcggttcctgcccaaccctgccggcgtgcagctggaagatcctgagttccaggcctccaacatcatgcactccatcaatggctatgtgttcgacagcctgcagctgagcgtgtgcctgcacgaggtggcctactggtacatcctgagcatcggggcccagaccgacttcctgtccgtgttcttctccggctacaccttcaagcacaagatggtgtacgaggataccctgaccctgttcccctttagcggcgaaaccgtgttcatgagcatggaaaaccccggcctgtggatcctgggctgccacaacagcgacttccggaacagaggcatgaccgccctgctgaaggtgtccagctgcgacaagaacaccggcgactactacgaggacagctatgaggacatcagcgcctacctgctgagcaagaacaatgccatcgagcccagaagcttcagccagaacccccccgtgctgaagcggcaccagagagagatcacccggaccaccctgcagtccgaccaggaagagatcgattacgacgacaccatcagcgtggaaatgaagaaagaagatttcgacatctacgacgaggacgagaaccagagcccccggtcctttcagaaaaagacccggcactacttcattgccgctgtggaacggctgtgggactacggcatgagcagcagccctcacgtgctgagaaacagggcccagagcggcagcgtgccccagttcaagaaagtggtgttccaggaattcacagacggcagcttcacccagcctctgtaccgcggcgagctgaatgagcacctgggactgctgggcccctatatcagagccgaagtggaagataatatcatggtcaccttccggaatcaggcctcccggccctacagcttctacagctccctgatcagctacgaagaggaccagagacagggcgctgagccccggaagaacttcgtgaagcccaacgagactaagacctacttttggaaggtgcagcaccacatggcccctacaaaggacgagttcgactgcaaggcctgggcctacttctccgatgtggacctggaaaaggacgtgcactctgggctgatcggccccctgctcgtgtgccacaccaacaccctgaatcccgcccacggcagacaagtgacagtgcaggaattcgccctgttcttcaccatcttcgacgaaacaaagagctggtacttcaccgaaaacatggaaagaaactgccgggctccctgcaacatccagatggaagatcccaccttcaaagagaactaccggttccacgccatcaacggctacatcatggacacactgcccggcctcgtgatggctcaggatcagcggatccggtggtatctgctgtccatgggctccaacgagaacatccacagcatccacttcagcggccacgtgttcaccgtgcggaaaaaagaagagtacaaaatggccctgtacaacctgtaccctggggtgttcgagacagtggaaatgctgcccagcaaggccggcatctggcgggtggaatgtctgatcggcgagcatctgcacgctgggatgagcacactgtttctggtgtacagcaacaagtgccagacacctctgggcatggcctctggccacatccgggactttcagatcacagccagcggccagtatggccagtgggccccaaaactggccagactgcactacagcggcagcatcaacgcctggtccaccaaagagcccttcagctggatcaaggtggacctgctggctcccatgatcatccacggaatcaagacccagggcgccagacagaagttcagcagcctgtacatcagccagttcatcatcatgtacagcctggacggcaagaagtggcagacctaccggggcaatagcaccggcaccctgatggtgttcttcggcaacgtggactccagcggcattaagcacaacatcttcaacccccccatcattgcccggtacatccggctgcaccccacccactacagcatccggtccaccctgagaatggaactgatgggctgcgacctgaactcctgcagcatgcccctggggatggaaagcaaggccatctccgacgcccagatcaccgcctccagctacttcaccaacatgttcgccacctggtccccatccaaggcccggctgcatctgcagggcagaagcaatgcttggaggccccaagtgaacaaccccaaagaatggctgcaggtggacttccagaaaaccatgaaagtgaccggcgtgaccacccagggcgtgaagtctctgctgacctctatgtacgtgaaagagttcctgatctccagcagccaggacggccaccagtggaccctgtttttccagaacggcaaagtgaaagtgtttcaggggaaccaggactccttcacccccgtcgtgaatagcctggaccctccactgctgaccagatacctgcggatccaccctcagagttgggtgcaccagattgctctgcggatggaagtgctgggatgcgaggcccaggacctgtactgacactagtaataaaagatcagagctgtagagatctgtgtgttggttttttgtgtgcggccggtaccaggaacccctagtgatggagttggccactccctctctgcgcgctcgctcgctcactgaggccgggcgaccaaaggtcgcccgacgcccgggctttgcccgggcggcctcagtgagcgagcgagcgcgcagagagggagtggcc

SEQ ID NO: 2 - DNA, 229 bp, Artificial Sequence
  Synthetic Construct
tgtctgtctgcacatttcgtagagcgagtgttccgatactctaatctcccggggcaaaggtcgtattgacttaggttacttattctccttttgttgactaagtcaataatcagaatcagcaggtttggagtcagcttggcagggatcagcagcctgggttggaaggagggggtataaaagccccttcaccaggagaagccgtcacacagatccacaagctcctgctagc

SEQ ID NO: 3 - DNA, 341 bp, Artificial Sequence
  Synthetic Construct
ctacctgctgatcgcccggcccctgttcaaacatgtcctaatactctgtcggggcaaaggtcggcagtagttttccatcttactcaacatcctcccagtgtacgtaggatcctgtctgtctgcacatttcgtagagcgagtgttccgatactctaatctcccggggcaaaggtcgtattgacttaggttacttattctccttttgttgactaagtcaataatcagaatcagcaggtttggagtcagcttggcagggatcagcagcctgggttggaaggagggggtataaaagccccttcaccaggagaagccgtcacacagatccacaagctcctgctagc

SEQ ID NO: 4 - DNA, 13524 bp, Artificial Sequence
  Synthetic Construct
gaatgcaattgttgttgttaacttgtttattgcagcttataatggttacaaataaagcaatagcatcacaaatttcacaaataaagcatttttttcactgcattctagttgtggtttgtccaaactcatcaatgtatcttatcatgtctggatccgctagaactaggaattcgctagcggtaccgatatcctagtggatcccccgtacacaggaagtgacaattttcgcgcggttttaggcggatgttgtagtaaatttgggcgtaaccgagtaagatttgggtggtcacgctgggtatttaagcccgagtgagcacgcagggtctccattttgaagcgggaggtttgaacgcgcagccgccatgccggggttttacgagattgtgattaaggtccccagcgaccttgacgagcatctgcccggcatttctgacagctttgtgaactgggtggccgagaaggaatgggagttgccgccagattctgacatggatctgaatctgattgagcaggcacccctgaccgtggccgagaagctgcagcgcgactttctgacggaatggcgccgtgtgagtaaggccccggaggcccttttctttgtgcaatttgagaagggagagagctacttccacatgcacgtgctcgtggaaaccaccggggtgaaatccatggttttgggacgtttcctgagtcagattcgcgaaaaactgattcagagaatttaccgcgggatcgagccgactttgccaaactggttcgcggtcacaaagaccagaaatggcgccggaggcgggaacaaggtggtggatgagtgctacatccccaattacttgctccccaaaacccagcctgagctccagtgggcgtggactaatatggaacagtatttaagcgcctgtttgaatctcacggagcgtaaacggttggtggcgcagcatctgacgcacgtgtcgcagacgcaggagcagaacaaagagaatcagaatcccaattctgatgcgccggtgatcagatcaaaaacttcagccaggtacatggagctggtcgggtggctcgtggacaaggggattacctcggagaagcagtggatccaggaggaccaggcctcatacatctccttcaatgcggcctccaactcgcggtcccaaatcaaggctgccttggacaatgcgggaaagattatgagcctgactaaaaccgcccccgactacctggtgggccagcagcccgtggaggacatttccagcaatcggatttataaaattttggaactaaacgggtacgatccccaatatgcggcttccgtctttctgggatgggccacgaaaaagttcggcaagaggaacaccatctggctgtttgggcctgcaactaccgggaagaccaacatcgcggaggccatagcccacactgtgcccttctacgggtgcgtaaactggaccaatgagaactttcccttcaacgactgtgtcgacaagatggtgatctggtgggaggaggggaagatgaccgccaaggtcgtggagtcggccaaagccattctcggaggaagcaaggtgcgcgtggaccagaaatgcaagtcctcggcccagatagacccgactcccgtgatcgtcacctccaacaccaacatgtgcgccgtgattgacgggaactcaacgaccttcgaacaccagcagccgttgcaagaccggatgttcaaatttgaactcacccgccgtctggatcatgactttgggaaggtcaccaagcaggaagtcaaagactttttccggtgggcaaaggatcacgtggttgaggtggagcatgaattctacgtcaaaaagggtggagccaagaaaagacccgcccccagtgacgcagatataagtgagcccaaacgggtgcgcgagtcagttgcgcagccatcgacgtcagacgcggaagcttcgatcaactacgcagacaggtaccaaaacaaatgttctcgtcacgtgggcatgaatctgatgctgtttccctgcagacaatgcgagagaatgaatcagaattcaaatatctgcttcactcacggacagaaagactgtttagagtgctttcccgtgtcagaatctcaacccgtttctgtcgtcaaaaaggcgtatcagaaactgtgctacattcatcatatcatgggaaaggtgccagacgcttgcactgcctgcgatctggtcaatgtggatttggatgactgcatctttgaacaataaatgatttaaatcaggtatggctgccgatggttatcttccagattggctcgaggacaacctctctgagggcattcgcgagtggtgggacctgaaacctggagccccgaaacccaaagccaaccagcaaaagcaggacgacggccggggtctggtgcttcctggctacaagtacctcggacccttcaacggactcgacaagggggagcccgtcaacgcggcggacgcagcggccctcgagcacgacaaggcctacgaccagcagctcaaagcgggtgacaatccgtacctgcggtataaccacgccgacgccgagtttcaggagcgtctgcaagaagatacgtcttttgggggcaacctcgggcgagcagtcttccaggccaagaagcgggttctcgaacctctcggtctggttgaggaaggcgctaagacggctcctggaaagaagagaccggtagagcagtcaccccaagaaccagactcatcctcgggcatcggcaaatcaggccagcagcccgctaaaaagagactcaattttggtcagactggcgactcagagtcagtccccgacccacaacctctcggagaacctccagaagccccctcaggtctgggacctaatacaatggcttcaggcggtggcgctccaatggcagacaataacgaaggcgccgacggagtgggtaattcctcgggaaattggcattgcgattccacatggctgggggacagagtcatcaccaccagcacccgaacctgggcattgcccacctacaacaaccacctctacaagcaaatctccaatggaacatcgggaggaagcaccaacgacaacacctactttggctacagcaccccctgggggtattttgacttcaacagattccactgccacttctcaccacgtgactggcagcgactcatcaacaacaactggggattccggccaaagagactcaacttcaagctgttcaacatccaggtcaaggaggttacgacgaacgaaggcaccaagaccatcgccaataaccttaccagcaccgtccaggtctttacggactcggagtaccagctaccgtacgtcctaggctctgcccaccaaggatgcctgccaccgtttcctgcagacgtcttcatggttcctcagtacggctacctgacgctcaacaatggaagtcaagcgttaggacgttcttctttctactgtctggaatacttcccttctcagatgctgagaaccggcaacaactttcagttcagctacactttcgaggacgtgcctttccacagcagctacgcacacagccagagtctagatcgactgatgaaccccctcatcgaccagtacctatactacctggtcagaacacagacaactggaactgggggaactcaaactttggcattcagccaagcaggccctagctcaatggccaatcaggctagaaactgggtacccgggccttgctaccgtcagcagcgcgtctccacaaccaccaaccaaaataacaacagcaactttgcgtggacgggagctgctaaattcaagctgaacgggagagactcgctaatgaatcctggcgtggctatggcatcgcacaaagacgacgaggaccgcttctttccatcaagtggcgttctcatatttggcaagcaaggagccgggaacgatggagtcgactacagccaggtgctgattacagatgaggaagaaattaaagccaccaaccctgtagccacagaggaatacggagcagtggccatcaacaaccaggccgctaacacgcaggcgcaaactggacttgtgcataaccagggagttattcctggtatggtctggcagaaccgggacgtgtacctgcagggccctatttgggctaaaatacctcacacagatggcaactttcacccgtctcctctgatgggtggatttggactgaaacacccacctccacagattctaattaaaaatacaccagtgccggcagatcctcctcttaccttcaatcaagccaagctgaactctttcatcacgcagtacagcacgggacaagtcagcgtggaaatcgagtgggagctgcagaaagaaaacagcaagcgctggaatccagagatccagtatacttcaaactactacaaatctacaaatgtggactttgctgtcaataccgaaggtgtttactctgagcctcgccccattggtactcgttacctcacccgtaatttgtaattgcctgttaatcaataaaccggttaattcgtttcagttgaactttggtctctgcgggccggccttaattaacatgtgagcaaaaggccagcaaaaggccaggaaccgtaaaaaggccgcgttgctggcgtttttccataggctccgcccccctgacgagcatcacaaaaatcgacgctcaagtcagaggtggcgaaacccgacaggactataaagataccaggcgtttccccctggaagctccctcgtgcgctctcctgttccgaccctgccgcttaccggatacctgtccgcctttctcccttcgggaagcgtggcgctttctcatagctcacgctgtaggtatctcagttcggtgtaggtcgttcgctccaagctgggctgtgtgcacgaaccccccgttcagcccgaccgctgcgccttatccggtaactatcgtcttgagtccaacccggtaagacacgacttatcgccactggcagtagccactggtaacaggattagcagagcgaggtatgtaggcggtgctacagagttcttgaagtggtggcctaactacggctacactagaagaacagtatttggtatctgcgctctgctgaagccagttaccttcggaaaaagagttggtagctcttgatccggcaaacaaaccaccgctggtagcggtggtttttttgtttgcaagcagcagattacgcgcagaaaaaaaggatctcaagaagatcctttgatcttttctacggggtctgacgctcagtggaacgaaaactcacgttaagggattttggtcatgagattatcaaaaaggatcttcacctagatccttttcacgtagaaagccagtccgcagaaacggtgctgaccccggatgaatgtcagctactgggctatctggacaagggaaaacgcaagcgcaaagagaaagcaggtagcttgcagtgggcttacatggcgatagctagactgggcggttttatggacagcaagcgaaccggaattgccagctggggcgccctctggtaaggttgggaagccctgcaaagtaaactggatggctttcttgccgccaaggatctgatggcgcaggggatcaagatccgatcaagagacaggatgaggatcgtttcgcatgattgaacaagatggattgcacgcaggttctccggccgcttgggtggagaggctattcggctatgactgggcacaacagacaatcggctgctctgatgccgccgtgttccggctgtcagcgcaggggcgcctggttctttttgtcaagaccgacctgtccggtgccctgaatgaactgcaagacgaggcagcgcggctatcgtggctggccacgacgggcgttccttgcgcagctgtgctcgacgttgtcactgaagcgggaagggactggctgctattgggcgaagtgccggggcaggatctcctgtcatctcaccttgctcctgccgagaaagtatccatcatggctgatgcaatgcggcggctgcatacgcttgatccggctacctgcccattcgaccaccaagcgaaacatcgcatcgagcgagcacgtactcggatggaagccggtcttgtcgatcaggatgatctggacgaagagcatcaggggctcgcgccagccgaactgttcgccaggctcaaggcgagcatgcccgacggcgaggatctcgtcgtgacccatggcgatgcctgcttgccgaatatcatggtggaaaatggccgcttttctggattcatcgactgtggccggctgggtgtggcggaccgctatcaggacatagcgttggctacccgtgatattgctgaagagcttggcggcgaatgggctgaccgcttcctcgtgctttacggtatcgccgctcccgattcgcagcgcatcgccttctatcgccttcttgacgagttcttctgaattaattaagcggccgctcatgagcggatacatatttgaatgtatttagaaaaataaacaaataggggttccgcgcacatttccccgaaaagtgccacctgacgtcagatccggtgcgggcctcttcgctattacgccagctggcgaaagggggatgtgctgcaaggcgattaagttgggtaacgccagggttttcccagtcacgacgttgtaaaacgacggccagtgaattcgcgagctcttggccactccctctctgcgcgctcgctcgctcactgaggccgggcgaccaaaggtcgcccgacgcccgggctttgcccgggcggcctcagtgagcgagcgagcgcgcagagagggagtggccaactccatcactaggggttcctacgcgtgtctgtctgcacatttcgtagagcgagtgttccgatactctaatctccctaggcaaggttcatatttgtgtaggttacttattctccttttgttgactaagtcaataatcagaatcagcaggtttggagtcagcttggcagggatcagcagcctgggttggaaggagggggtataaaagccccttcaccaggagaagccgtcacacagatccacaagctcctgctagcaggtaagtgccgtgtgtggttcccgcgggcctggcctctttacgggttatggcccttgcgtgccttgaattactgacactgacatccactttttctttttctccacaggtatcgattctctagagccaccatgcagatcgagctgtctacctgcttcttcctgtgcctgctgcggttctgcttcagcgccaccagacggtactatctgggcgccgtggaactgagctgggactacatgcagagcgacctgggcgagctgcccgtggatgccagattccctccaagagtgcccaagagcttccccttcaacacctccgtggtgtacaagaaaaccctgttcgtggaattcaccgaccacctgttcaatatcgccaagcccagacccccctggatgggcctgctgggacctacaattcaggccgaggtgtacgacaccgtcgtgatcaccctgaagaacatggccagccaccccgtgtctctgcatgccgtgggagtgtcctactggaaggcctctgagggcgccgagtacgacgatcagaccagccagcgcgagaaagaggacgacaaggtgttccctggcggcagccacacctacgtgtggcaggtgctgaaagaaaacggccccatggcctccgaccctctgtgcctgacatacagctacctgagccacgtggacctcgtgaaggacctgaacagcggcctgatcggagccctgctcgtgtgtagagagggcagcctggccaaagagaaaacccagaccctgcacaagttcatcctgctgttcgccgtgttcgacgagggcaagagctggcacagcgagacaaagaacagcctgatgcaggaccgggacgccgcctctgctagagcctggcccaaaatgcacaccgtgaacggctacgtgaacagaagcctgcccggactgatcggctgccaccggaagtctgtgtactggcacgtgatcggcatgggcaccacccctgaggtgcacagcatctttctggaaggacacacctttctcgtgcggaaccaccggcaggccagcctggaaatcagccctatcaccttcctgaccgcccagacactgctgatggacctgggccagtttctgctgttctgccacatcagctcccaccagcacgacggcatggaagcctacgtgaaggtggacagctgccccgaggaaccccagctgcggatgaagaacaacgaggaagccgaggactacgacgacgacctgaccgacagcgagatggacgtggtgcgcttcgacgacgataacagccccagcttcatccagatcagaagcgtggccaagaagcaccccaagacctgggtgcactatatcgccgccgaggaagaggactgggattacgcccctctggtgctggcccccgacgacagaagctacaagagccagtacctgaacaatggcccccagcggatcggccggaagtataagaaagtgcggttcatggcctacaccgacgagacattcaagaccagagaggccatccagcacgagagcggcatcctgggccctctgctgtatggcgaagtgggcgacaccctgctgatcatcttcaagaaccaggccagcagaccctacaacatctaccctcacggcatcaccgacgtgcggcccctgtactccagaaggctgcccaagggcgtgaaacacctgaaggacttccccatcctgcccggcgagatcttcaagtacaagtggaccgtgaccgtggaagatggccccaccaagagcgaccccagatgcctgacacggtactacagcagcttcgtgaacatggaacgggacctggcctccggcctgattggcccactgctgatctgctacaaagaaagcgtggaccagcggggcaaccagatcatgagcgacaagcggaacgtgatcctgtttagcgtgttcgatgagaaccggtcctggtatctgaccgagaatatccagcggttcctgcccaaccctgccggcgtgcagctggaagatcctgagttccaggcctccaacatcatgcactccatcaatggctatgtgttcgacagcctgcagctgagcgtgtgcctgcacgaggtggcctactggtacatcctgagcatcggggcccagaccgacttcctgtccgtgttcttctccggctacaccttcaagcacaagatggtgtacgaggataccctgaccctgttcccctttagcggcgaaaccgtgttcatgagcatggaaaaccccggcctgtggatcctgggctgccacaacagcgacttccggaacagaggcatgaccgccctgctgaaggtgtccagctgcgacaagaacaccggcgactactacgaggacagctatgaggacatcagcgcctacctgctgagcaagaacaatgccatcgagcccagaagcttcagccagaacccccccgtgctgaagcggcaccagagagagatcacccggaccaccctgcagtccgaccaggaagagatcgattacgacgacaccatcagcgtggaaatgaagaaagaagatttcgacatctacgacgaggacgagaaccagagcccccggtcctttcagaaaaagacccggcactacttcattgccgctgtggaacggctgtgggactacggcatgagcagcagccctcacgtgctgagaaacagggcccagagcggcagcgtgccccagttcaagaaagtggtgttccaggaattcacagacggcagcttcacccagcctctgtaccgcggcgagctgaatgagcacctgggactgctgggcccctatatcagagccgaagtggaagataatatcatggtcaccttccggaatcaggcctcccggccctacagcttctacagctccctgatcagctacgaagaggaccagagacagggcgctgagccccggaagaacttcgtgaagcccaacgagactaagacctacttttggaaggtgcagcaccacatggcccctacaaaggacgagttcgactgcaaggcctgggcctacttctccgatgtggacctggaaaaggacgtgcactctgggctgatcggccccctgctcgtgtgccacaccaacaccctgaatcccgcccacggcagacaagtgacagtgcaggaattcgccctgttcttcaccatcttcgacgaaacaaagagctggtacttcaccgaaaacatggaaagaaactgccgggctccctgcaacatccagatggaagatcccaccttcaaagagaactaccggttccacgccatcaacggctacatcatggacacactgcccggcctcgtgatggctcaggatcagcggatccggtggtatctgctgtccatgggctccaacgagaacatccacagcatccacttcagcggccacgtgttcaccgtgcggaaaaaagaagagtacaaaatggccctgtacaacctgtaccctggggtgttcgagacagtggaaatgctgcccagcaaggccggcatctggcgggtggaatgtctgatcggcgagcatctgcacgctgggatgagcacactgtttctggtgtacagcaacaagtgccagacacctctgggcatggcctctggccacatccgggactttcagatcacagccagcggccagtatggccagtgggccccaaaactggccagactgcactacagcggcagcatcaacgcctggtccaccaaagagcccttcagctggatcaaggtggacctgctggctcccatgatcatccacggaatcaagacccagggcgccagacagaagttcagcagcctgtacatcagccagttcatcatcatgtacagcctggacggcaagaagtggcagacctaccggggcaatagcaccggcaccctgatggtgttcttcggcaacgtggactccagcggcattaagcacaacatcttcaacccccccatcattgcccggtacatccggctgcaccccacccactacagcatccggtccaccctgagaatggaactgatgggctgcgacctgaactcctgcagcatgcccctggggatggaaagcaaggccatctccgacgcccagatcaccgcctccagctacttcaccaacatgttcgccacctggtccccatccaaggcccggctgcatctgcagggcagaagcaatgcttggaggccccaagtgaacaaccccaaagaatggctgcaggtggacttccagaaaaccatgaaagtgaccggcgtgaccacccagggcgtgaagtctctgctgacctctatgtacgtgaaagagttcctgatctccagcagccaggacggccaccagtggaccctgtttttccagaacggcaaagtgaaagtgtttcaggggaaccaggactccttcacccccgtcgtgaatagcctggaccctccactgctgaccagatacctgcggatccaccctcagagttgggtgcaccagattgctctgcggatggaagtgctgggatgcgaggcccaggacctgtactgacaactagtaataaaagatcagagctgtagagatctgtgtgttggttttttgtgtgcggccggtacccaggaacccctagtgatggagttggccactccctctctgcgcgctcgctcgctcactgaggccgggcgaccaaaggtcgcccgacgcccgggctttggtcgggcggcctcagtgagcgagcgagcgcgcagagagggagtggccggaagcttggcgtaatcatggtcatagctgtttcctgtgtgaaattgttatccgctcacaattccacacaacatacgagccggaagcataaagtgtaaagcctggggtgcctaatgagtgagctaactcacattaattgcgttgcgctcactgcccgctttccagtcgggaaacctgtcgtgccagctgcattaatgaatcggccaacgcgcggggagaggcggtttgcgtattgggcgctcttccgctgatctcatactagcgaacgccagcaagacgtagcccagcgcgtcggccccgagatgcgccgcgtgcggctgctggagatggcggacgcgatggatatgttctgccaagggttggtttgcgcattcacagttctccgcaagaattgattggctccaattcttggagtggtgaatccgttagcgaggtgccgccctgcttcatccccgtggcccgttgctcgcgtttgctggcggtgtccccggaagaaatatatttgcatgtctttagttctatgatgacacaaaccccgcccagcgtcttgtcattggcgaattccggctgtggaatgtgtgtcagttagggtgtggaaagtccccaggctccccagcaggcagaagtatgcaaagcatgcatctcaattagtcagcaaccaggtgtggaaagtccccaggctccccagcaggcagaagtatgcaaagcatgcatctcaattagtcagcaaccatagtcccgcccctaactccgcccatcccgcccctaactccgcccagttccgcccattctccgccccatggctgactaattttttttatttatgcagaggccgaggccgcctcggcctctgagctattccagaagtagtgaggaggcttttttggaggcctaggcttttgcaaaaagcttgcatgcctgcaggtcggccgccacgaccggtgccgccaccatcccctgacccacgcccctgacccctcacaaggagacgaccttccatgaccgagtacaagcccacggtgcgcctcgccacccgcgacgacgtcccccgggccgtacgcaccctcgccgccgcgttcgccgactaccccgccacgcgccacaccgtcgacccggaccgccacatcgagcgggtcaccgagctgcaagaactcttcctcacgcgcgtcgggctcgacatcggcaaggtgtgggtcgcggacgacggcgccgcggtggcggtctggaccacgccggagagcgtcgaagcgggggcggtgttcgccgagatcggcccgcgcatggccgagttgagcggttcccggctggccgcgcagcaacagatggaaggcctcctggcgccgcaccggcccaaggagcccgcgtggttcctggccaccgtcggcgtctcgcccgaccaccagggcaagggtctgggcagcgccgtcgtgctccccggagtggaggcggccgagcgcgccggggtgcccgccttcctggagacctccgcgccccgcaacctccccttctacgagcggctcggcttcaccgtcaccgccgacgtcgaggtgcccgaaggaccgcgcacctggtgcatgacccgcaagcccggtgcctgacgcccgccccacgacccgcagcgcccgaccgaaaggagcgcacgaccccatggctccgaccgaagccacccggggcggccccgccgaccccgcacccgcccccgaggcccaccgactctagaggatcataatcagccataccacatttgtagaggttttacttgctttaaaaaacctcccacacctccccctgaacctgaaacataaaat

SEQ ID NO: 5 - DNA, 17 bp, Artificial Sequence
  Synthetic Construct
gacgtggtgcgcttcga

SEQ ID NO: 6 - DNA, 20 bp, Artificial Sequence
  Synthetic Construct
gggcgtaatcccagtcctct

SEQ ID NO: 7 - DNA, 22 bp, Artificial Sequence
  Synthetic Construct
aagcgtggccaagaagcacccc

SEQ ID NO: 8 - DNA, 21 bp, Artificial Sequence
  Synthetic Construct
gttgccattgctacaggcatc

SEQ ID NO: 9 - DNA, 19 bp, Artificial Sequence
  Synthetic Construct
actcgccttgatcgttggg

SEQ ID NO: 10 - DNA, 28 bp, Artificial Sequence
  Synthetic Construct
acgctcgtcgtttggtatggcttcattc

SEQ ID NO: 11 - DNA, 17 bp, Artificial Sequence
  Synthetic Construct
ggaccgccacatcgagc

SEQ ID NO: 12 - DNA, 15 bp, Artificial Sequence
  Synthetic Construct
ccccgcttcgacgct

SEQ ID NO: 13 - DNA, 28 bp, Artificial Sequence
  Synthetic Construct
tcaccgagctgcaagaactcttcctcac

SEQ ID NO: 14 - DNA, 23 bp, Artificial Sequence
  Synthetic Construct
gaccaggcctcatacatctcctt

SEQ ID NO: 15 - DNA, 18 bp, Artificial Sequence
  Synthetic Construct
ggcagccttgatttggga

SEQ ID NO: 16 - DNA, 20 bp, Artificial Sequence
  Synthetic Construct
aatgcggcctccaactcgcg

SEQ ID NO: 17 - DNA, 19 bp, Artificial Sequence
  Synthetic Construct
caacacggcgaccctacaa

SEQ ID NO: 18 - DNA, 28 bp, Artificial Sequence
  Synthetic Construct
tccaatactgtcttgcaatatacacagg

SEQ ID NO: 19 - DNA, 28 bp, Artificial Sequence
  Synthetic Construct
tgcacggaactgaacacttcactgcaag

SEQ ID NO: 20 - DNA, 24 bp, Artificial Sequence
  Synthetic Construct
ccgtcgtgaatagcctggaccctc

SEQ ID NO: 21 - DNA, 28 bp, Artificial Sequence
  Synthetic Construct
atctgtgtgttggttttttgtgtgcggc

SEQ ID NO: 22 - DNA, 29 bp, Artificial Sequence
  Synthetic Construct
aatcccagtcctcttcctcggcggcgata

SEQ ID NO: 23 - DNA, 29 bp, Artificial Sequence
  Synthetic Construct
agtatcggaacactcgctctacgaaatgt

SEQ ID NO: 24 - DNA, 78 bp, Artificial Sequence
  Synthetic Construct
cactccctctctgcgcgctcgctcgctcactgaggccgggcgaccaaaggtcgcccacgcccgggctttgcccgggcg